European Patent Specification EP 3 256 579 B1, published August 30, 2023. Title: CYSTEINE PROTEASE. Applicant: HANSA MEDICAL AB. The sequence listing filed with the application follows.

SEQUENCE LISTING (55 sequences)

SEQ ID NO: 1 - protein, 339 aa, Streptococcus pyogenes
MRKRCYSTSAAVLAAVTLFVLSVDRGVIADSFSANQEIRYSEVTPYHVTSVWTKGVTPPANFTQGEDVFHAPYVANQGWYDITKTFNGKDDLLCGAATAGNMLHWWFDQNKDQIKRYLEEHPEKQKINFNGEQMFDVKEAIDTKNHQLDSKLFEYFKEKAFPYLSTKHLGVFPDHVIDMFINGYRLSLTNHGPTPVKEGSKDPRGGIFDAVFTRGDQSKLLTSRHDFKEKNLKEISDLIKKELTEGKALGLSHTYANVRINHVINLWGADFDSNGNLKAIYVTDSDSNASIGMKKYFVGVNSAGKVAISAKEIKEDNIGAQVLGLFTLSTGQDSWNQTN

SEQ ID NO: 2 - protein, 310 aa, Streptococcus pyogenes
DSFSANQEIRYSEVTPYHVTSVWTKGVTPPANFTQGEDVFHAPYVANQGWYDITKTFNGKDDLLCGAATAGNMLHWWFDQNKDQIKRYLEEHPEKQKINFNGEQMFDVKEAIDTKNHQLDSKLFEYFKEKAFPYLSTKHLGVFPDHVIDMFINGYRLSLTNHGPTPVKEGSKDPRGGIFDAVFTRGDQSKLLTSRHDFKEKNLKEISDLIKKELTEGKALGLSHTYANVRINHVINLWGADFDSNGNLKAIYVTDSDSNASIGMKKYFVGVNSAGKVAISAKEIKEDNIGAQVLGLFTLSTGQDSWNQTN

SEQ ID NO: 3 - protein, 349 aa, Streptococcus pyogenes
MKTIAYPNKPHSLSAGLLTAIAIFSLASSNITYADDYQRNATEAYAKEVPHQITSVWTKGVTPLTPEQFRYNNEDVIHAPYLAHQGWYDITKAFDGKDNLLCGAATAGNMLHWWFDQNKTEIEAYLSKHPEKQKIIFNNQELFDLKAAIDTKDSQTNSQLFNYFRDKAFPNLSARQLGVMPDLVLDMFINGYYLNVFKTQSTDVNRPYQDKDKRGGIFDAVFTRGDQTTLLTARHDLKNKGLNDISTIIKQELTEGRALALSHTYANVSISHVINLWGADFNAEGNLEAIYVTDSDANASIGMKKYFVGINAHGHVAISAKKIEGENIGAQVLGLFTLSSGKDIWQKLS

SEQ ID NO: 4 - protein, 315 aa, Streptococcus pyogenes
DDYQRNATEAYAKEVPHQITSVWTKGVTPLTPEQFRYNNEDVIHAPYLAHQGWYDITKAFDGKDNLLCGAATAGNMLHWWFDQNKTEIEAYLSKHPEKQKIIFNNQELFDLKAAIDTKDSQTNSQLFNYFRDKAFPNLSARQLGVMPDLVLDMFINGYYLNVFKTQSTDVNRPYQDKDKRGGIFDAVFTRGDQTTLLTARHDLKNKGLNDISTIIKQELTEGRALALSHTYANVSISHVINLWGADFNAEGNLEAIYVTDSDANASIGMKKYFVGINAHGHVAISAKKIEGENIGAQVLGLFTLSSGKDIWQKLS

SEQ ID NO: 5 - protein, 313 aa, Streptococcus pyogenes
DDYQRNATEAYAKEVPHQITSVWTKGVTPLTPEQFRYNNEDVFHAPYVANQGWYDITKAFDGKDNLLCGAATAGNMLHWWFDQNKDQIKRYLEEHPEKQKINFNGDNMFDVKKAIDTKNHQLDSKLFNYFKEKAFPGLSARRIGVFPDHVIDMFINGYRLSLTNHGPTPVKEGSKDPRGGIFDAVFTRGNQSKLLTSRHDFKNKNLNDISTIIKQELTKGKALGLSHTYANVSINHVINLWGADFNAEGNLEAIYVTDSDSNASIGMKKYFVGVNAHGHVAISAKKIEGENIGAQVLGLFTLSTGQDSWQKLS

SEQ ID NO: 6 - protein, 315 aa, Streptococcus pyogenes
DDYQRNATEAYAKEVPHQITSVWTKGVTPLTPEQFRYNNEDVIHAPYLANQGWYDITKAFDGKDNLLCGAATAGNMLHWWFDQNKTEIEAYLSKHPEKQKIIFRNQELFDLKEAIRTKDSQTNSQLFEYFRDKAFPYLSARQLGVMPDLVLDMFINGYYLNVFKTQSTDVKRPYQDKDKRGGIFDAVFTRGNQTTLLTARHDLKNKGLNDISTIIKEELTKGRALALSHTYANVSISHVINLWGADFNAEGNLEAIYVTDSDANASIGMKKYFVGINKHGHVAISAKKIEGENIGAQVLGLFTLSSGKDIWQKLN

SEQ ID NO: 7 - protein, 315 aa, Streptococcus pyogenes
DDYQRNATEAYAKEVPHQITSVWTKGVTPLTPEQFRYNNEDVIHAPYLAHQGWYDITKTFNGKDNLLCGAATAGNMLHWWFDQNKTEIEAYLSKHPEKQKIIFNNEELFDLKAAIDTKDSQTNSQLFNYFKEKAFPNLSTRQLGVMPDLVLDMFINGYYLNVFKTQSTDVNRPYQDKDKRGGIFDAVFTRGNQTTLLTARHDFKEKGLKDISTIIKQELTEGRALALSHTYANVSISHVINLWGADFDAEGNLKAIYVTDSDANASIGMKKYFVGINAHGKVAISAKKIEGENIGAQVLGLFTLSSGKDIWQQLS

SEQ ID NO: 8 - protein, 315 aa, Streptococcus pyogenes
DSFSANQEIRYSEVTPYHVTSVWTKGVTPLTPEQFRYNNEDVIHAPYLAHQGWYDITKAFDGKDNLLCGAATAGNMLHWWFDQNKTEIEAYLSKHPEKQKIIFNNQELFDLKAAIDTKDSQTNSQLFNYFRDKAFPNLSARQLGVMPDLVLDMFINGYYLNVFKTQSTDVNRPYQDKDKRGGIFDAVFTRGDQTTLLTARHDLKNKGLNDISTIIKQELTEGRALALSHTYANVSISHVINLWGADFNAEGNLEAIYVTDSDANASIGMKKYFVGINAHGHVAISAKKIEGENIGAQVLGLFTLSSGKDIWQKLS

SEQ ID NO: 9 - protein, 295 aa, Streptococcus pyogenes
SVWTKGVTPLTPEQFRYNNEDVIHAPYLAHQGWYDITKAFDGKDNLLCGAATAGNMLHWWFDQNKTEIEAYLSKHPEKQKIIFNNQELFDLKAAIDTKDSQTNSQLFNYFRDKAFPNLSARQLGVMPDLVLDMFINGYYLNVFKTQSTDVNRPYQDKDKRGGIFDAVFTRGDQTTLLTARHDLKNKGLNDISTIIKQELTEGRALALSHTYANVSISHVINLWGADFNAEGNLEAIYVTDSDANASIGMKKYFVGINAHGHVAISAKKIEGENIGAQVLGLFTLSSGKDIWQKLS

SEQ ID NO: 10 - protein, 314 aa, Streptococcus pyogenes
DDYQRNATEAYAKEVPHQITSVWTKGVTPLTPEQFTQGEDVIHAPYLAHQGWYDITKAFDGKDNLLCGAATAGNMLHWWFDQNKTEIEAYLSKHPEKQKIIFNNQELFDLKAAIDTKDSQTNSQLFNYFRDKAFPNLSARQLGVMPDLVLDMFINGYYLNVFKTQSTDVNRPYQDKDKRGGIFDAVFTRGDQTTLLTARHDLKNKGLNDISTIIKQELTEGRALALSHTYANVSISHVINLWGADFNAEGNLEAIYVTDSDANASIGMKKYFVGINAHGHVAISAKKIEGENIGAQVLGLFTLSSGKDIWQKLS

SEQ ID NO: 11 - protein, 312 aa, Streptococcus pyogenes
DDYQRNATEAYAKEVPHQITSVWTKGVTPPEQFTQGEDVIHAPYLAHQGWYDITKAFDGKDNLLCGAATAGNMLHWWFDQNKTEIEAYLSKHPEKQKIIFNNQELFDLKAAIDTKDSQTNSQLFNYFRDKAFPNLSARQLGVMPDLVLDMFINGYYLNVFKTQSTDVNRPYQDKDKRGGIFDAVFTRGDQTTLLTARHDLKNKGLNDISTIIKQELTEGRALALSHTYANVSISHVINLWGADFNAEGNLEAIYVTDSDANASIGMKKYFVGINAHGHVAISAKKIEGENIGAQVLGLFTLSSGKDIWQKLS

SEQ ID NO: 12 - protein, 313 aa, Streptococcus pyogenes
DDYQRNATEAYAKEVPHQITSVWTKGVTPPEQFRYNNEDVIHAPYLAHQGWYDITKAFDGKDNLLCGAATAGNMLHWWFDQNKTEIEAYLSKHPEKQKIIFNNQELFDLKAAIDTKDSQTNSQLFNYFRDKAFPNLSARQLGVMPDLVLDMFINGYYLNVFKTQSTDVNRPYQDKDKRGGIFDAVFTRGDQTTLLTARHDLKNKGLNDISTIIKQELTEGRALALSHTYANVSISHVINLWGADFNAEGNLEAIYVTDSDANASIGMKKYFVGINAHGHVAISAKKIEGENIGAQVLGLFTLSSGKDIWQKLS

SEQ ID NO: 13 - protein, 312 aa, Streptococcus pyogenes
DDYQRNATEAYAKEVPHQITSVWTKGVTPPEQFTQGEDVIHAPYLAHQGWYDITKAFDGKDNLLCGAATAGNMLHWWFDQNKTEIEAYLSKHPEKQKIIINNQELFDLKAAIDTKDSQTNSQLFNYFRDKAFPNLSARQLGVMPDLVLDMFINGYYLNVFKTQSTDVNRPYQDKDKRGGIFDAVFTRGDQTTLLTARHDLKNKGLNDISTIIKQELTEGRALALSHTYANVSISHVINLWGADFNAEGNLEAIYVTDSDANASIGMKKYFVGINAHGHVAISAKKIEGENIGAQVLGLFTLSSGKDIWQKLS

SEQ ID NO: 14 - protein, 312 aa, Streptococcus pyogenes
DDYQRNATEAYAKEVPHQITSVWTKGVTPPEQFTQGEDVIHAPYLAHQGWYDITKAFDGKDNLLCGAATAGNMLHWWFDQNKTEIEAYLSKHPEKQKIIFRNQELFDLKAAIDTKDSQTNSQLFNYFRDKAFPNLSARQLGVMPDLVLDMFINGYYLNVFKTQSTDVNRPYQDKDKRGGIFDAVFTRGDQTTLLTARHDLKNKGLNDISTIIKQELTEGRALALSHTYANVSISHVINLWGADFNAEGNLEAIYVTDSDANASIGMKKYFVGINAHGHVAISAKKIEGENIGAQVLGLFTLSSGKDIWQKLS

SEQ ID NO: 15 - protein, 312 aa, Streptococcus pyogenes
DDYQRNATEAYAKEVPHQITSVWTKGVTPPEQFTQGEDVIHAPYLAHQGWYDITKAFDGKDNLLCGAATAGNMLHWWFDQNKTEIEAYLSKHPEKQKIIIRNQELFDLKAAIDTKDSQTNSQLFNYFRDKAFPNLSARQLGVMPDLVLDMFINGYYLNVFKTQSTDVNRPYQDKDKRGGIFDAVFTRGDQTTLLTARHDLKNKGLNDISTIIKQELTEGRALALSHTYANVSISHVINLWGADFNAEGNLEAIYVTDSDANASIGMKKYFVGINAHGHVAISAKKIEGENIGAQVLGLFTLSSGKDIWQKLS

SEQ ID NO: 16 - protein, 312 aa, Streptococcus pyogenes
DDYQRNATEAYAKEVPHQITSVWTKGVTPPEQFTQGEDVIHAPYLANQGWYDITKAFDGKDNLLCGAATAGNMLHWWFDQNKTEIEAYLSKHPEKQKIIFRNQELFDLKEAIRTKDSQTNSQLFEYFRDKAFPYLSARQLGVMPDLVLDMFINGYYLNVFKTQSTDVKRPYQDKDKRGGIFDAVFTRGNQTTLLTARHDLKNKGLNDISTIIKEELTKGRALALSHTYANVSISHVINLWGADFNAEGNLEAIYVTDSDANASIGMKKYFVGINKHGHVAISAKKIEGENIGAQVLGLFTLSSGKDIWQKLN

SEQ ID NO: 17 - protein, 292 aa, Streptococcus pyogenes
SVWTKGVTPPEQFTQGEDVIHAPYLAHQGWYDITKAFDGKDNLLCGAATAGNMLHWWFDQNKTEIEAYLSKHPEKQKIIFRNQELFDLKAAIDTKDSQTNSQLFNYFRDKAFPNLSARQLGVMPDLVLDMFINGYYLNVFKTQSTDVNRPYQDKDKRGGIFDAVFTRGNQTTLLTARHDLKNKGLNDISTIIKQELTEGRALALSHTYANVSISHVINLWGADFNAEGNLEAIYVTDSDANASIGMKKYFVGINAHGHVAISAKKIEGENIGAQVLGLFTLSSGKDIWQKLS

SEQ ID NO: 18 - protein, 312 aa, Streptococcus pyogenes
DDYQRNATEAYAKEVPHQITSVWTKGVTPPEQFTQGEDVIHAPYLAHQGWYDITKAFDGADNLLCGAATAGNMLHWWFDQNKTEIEAYLSKHPEKQKIIFRNQELFDLKAAIDTKDSQTNSQLFNYFRDKAFPNLSARQLGVMPDLVLDMFINGYYLNVFKTQSTDVNRPYQDKDKRGGIFDAVFTRGNQTTLLTARHDLKNKGLNDISTIIKQELTEGRALALSHTYANVSISHVINLWGADFNAEGNLEAIYVTDSDANASIGMKKYFVGINAHGHVAISAKKIEGENIGAQVLGLFTLSSGKDIWQKLS

SEQ ID NO: 19 - protein, 292 aa, Streptococcus pyogenes
SVWTKGVTPPEQFTQGEDVIHAPYLAHQGWYDITKAFDGADNLLCGAATAGNMLHWWFDQNKTEIEAYLSKHPEKQKIIFRNQELFDLKAAIDTKDSQTNSQLFNYFRDKAFPNLSARQLGVMPDLVLDMFINGYYLNVFKTQSTDVNRPYQDKDKRGGIFDAVFTRGNQTTLLTARHDLKNKGLNDISTIIKQELTEGRALALSHTYANVSISHVINLWGADFNAEGNLEAIYVTDSDANASIGMKKYFVGINAHGHVAISAKKIEGENIGAQVLGLFTLSSGKDIWQKLS

SEQ ID NO: 20 - protein, 312 aa, Streptococcus pyogenes
DDYQRNATEAYAKEVPHQITSVWTKGVTPPEQFTQGEDVIHAPYLAHQGWYDITKAFDGKDNLLCGAATAGNMLHWWFDQNKTEIEAYLSKHPEKQKIIFRNQELFDLKAAIDTKDSQTNSQLFNYFRDKAFPNLSARQLGVMPDLVLDMFINGYYLNVFKTQSTDVNRPYQDKDKRGGIFDAVFTRGNQTTLLTARHDLKNKGLNDISTIIKQELTEGRALALSHTYANVSISHVINLWGADFNAEGNLEAIYVTDSDANASIGMKKYFVGINAHGHVAISAKKIEGENIGAQVLGLFTLSSGKDIWQKLS

SEQ ID NO: 21 - protein, 312 aa, Streptococcus pyogenes
DDYQRNATEAYAKEVPHQITSVWTKGVTPLTPEQFTQGEDVFHAPYVANQGWYDITKAFDGKDNLLCGAATAGNMLHWWFDQNKDQIKRYLEEHPEKQKINFNGENMFDVKKAIDTKNHQLDSKLFNYFKEKAFPYLSAKHLGVFPDHVIDMFINGYRLSLTNHGPTPVKEGSKDPRGGIFDAVFTRGNQSKLLTSRHDFKNKNLNDISTIIKQELTKGKALGLSHTYANVRINHVINLWGADFNAEGNLEAIYVTDSDSNASIGMKKYFVGVNAHGHVAISAKKIEGENIGAQVLGLFTLSTGQDSWQKLS

SEQ ID NO: 22 - protein, 312 aa, Streptococcus pyogenes
DDYQRNATEAYAKEVPHQITSVWTKGVTPLTPEQFTQGEDVFHAPYVANQGWYDITKAFDGKDNLLCGAATAGNMLHWWFDQNKDQIKRYLEEHPEKQKINFRGENMFDVKEAIRTKNHQLDSKLFEYFKEKAFPYLSAKHLGVFPDHVIDMFINGYRLSLTNHGPTPVKKGSKDPRGGIFDAVFTRGNQSKLLTSRHDFKNKNLNDISTIIKSELTNGKALGLSHTYANVRINHVINLWGADFNAEGNLEAIYVTDSDSNASIGMKKYFVGVNKHGHVAISAKKIEGENIGAQVLGLFTLSTGQDSWQKLN

SEQ ID NO: 23 - protein, 312 aa, Streptococcus pyogenes
DDYQRNATEAYAKEVPHQITSVWTKGVTPLTPEQFTQGEDVFHAPYVANQGWYDITKTFNGKDDLLCGAATAGNMLHWWFDQNKDQIKRYLEEHPEKQKINFNGEQMFDVKEAIDTKNHQLDSKLFEYFKEKAFPYLSTKHLGVFPDHVIDMFINGYRLSLTNHGPTPVKEGSKDPRGGIFDAVFTRGNQSKLLTSRHDFKEKNLKEISDLIKQELTEGKALGLSHTYANVRINHVINLWGADFDAEGNLKAIYVTDSDSNASIGMKKYFVGVNAAGKVAISAKKIEGENIGAQVLGLFTLSTGQDSWNQTS

SEQ ID NO: 24 - protein, 312 aa, Streptococcus pyogenes
DDYQRNATEAYAKEVPHQITSVWTKGVTPLTPEQFTQGEDVFHAPYVANQGWYDITKTFNGKDDLLCGAATAGNMLHWWFDQNKDQIKRYLEEHPEKQKINFRGEQMFDVKEAIRTKNHQLDSKLFEYFKEKAFPYLSTKHLGVFPDHVIDMFINGYRLSLTNHGPTPVKKGSKDPRGGIFDAVFTRGNQSKLLTSRHDFKEKNLKEISDLIKEELTKGKALGLSHTYANVRINHVINLWGADFDAEGNLKAIYVTDSDSNASIGMKKYFVGVNKAGKVAISAKKIEGENIGAQVLGLFTLSTGQDSWNQTN

SEQ ID NO: 25 - protein, 310 aa, Streptococcus pyogenes
DDYQRNATEAYAKEVPHQITSVWTKGVTPPEQFTQGEDVIHAPYVANQGWYDITKAFDGKDNLLCGAATAGNMLHWWFDQNKDQIKRYLEEHPEKQKINFRGEQMFDVKKAIDTKNHQLDSKLFNYFKEKAFPGLSARRIGVFPDHVIDMFINGYRLSLTNHGPTPVKEGSKDPRGGIFDAVFTRGNQSKLLTSRHDFKNKNLNDISTIIKQELTKGKALGLSHTYANVSINHVINLWGADFNAEGNLEAIYVTDSDSNASIGMKKYFVGVNAHGHVAISAKKIEGENIGAQVLGLFTLSTGQDSWQKLS

SEQ ID NO: 26 - protein, 320 aa, Streptococcus pyogenes
MDSFSANQEIRYSEVTPYHVTSVWTKGVTPPANFTQGEDVFHAPYVANQGWYDITKTFNGKDDLLCGAATAGNMLHWWFDQNKDQIKRYLEEHPEKQKINFNGEQMFDVKEAIDTKNHQLDSKLFEYFKEKAFPYLSTKHLGVFPDHVIDMFINGYRLSLTNHGPTPVKEGSKDPRGGIFDAVFTRGDQSKLLTSRHDFKEKNLKEISDLIKKELTEGKALGLSHTYANVRINHVINLWGADFDSNGNLKAIYVTDSDSNASIGMKKYFVGVNSAGKVAISAKEIKEDNIGAQVLGLFTLSTGQDSWNQTNGGGHHHHHH

SEQ ID NO: 27 - protein, 325 aa, Streptococcus pyogenes
MDDYQRNATEAYAKEVPHQITSVWTKGVTPLTPEQFRYNNEDVIHAPYLAHQGWYDITKAFDGKDNLLCGAATAGNMLHWWFDQNKTEIEAYLSKHPEKQKIIFNNQELFDLKAAIDTKDSQTNSQLFNYFRDKAFPNLSARQLGVMPDLVLDMFINGYYLNVFKTQSTDVNRPYQDKDKRGGIFDAVFTRGDQTTLLTARHDLKNKGLNDISTIIKQELTEGRALALSHTYANVSISHVINLWGADFNAEGNLEAIYVTDSDANASIGMKKYFVGINAHGHVAISAKKIEGENIGAQVLGLFTLSSGKDIWQKLSGGGHHHHHH

SEQ ID NO: 28 - protein, 323 aa, Streptococcus pyogenes
MDDYQRNATEAYAKEVPHQITSVWTKGVTPLTPEQFRYNNEDVFHAPYVANQGWYDITKAFDGKDNLLCGAATAGNMLHWWFDQNKDQIKRYLEEHPEKQKINFNGDNMFDVKKAIDTKNHQLDSKLFNYFKEKAFPGLSARRIGVFPDHVIDMFINGYRLSLTNHGPTPVKEGSKDPRGGIFDAVFTRGNQSKLLTSRHDFKNKNLNDISTIIKQELTKGKALGLSHTYANVSINHVINLWGADFNAEGNLEAIYVTDSDSNASIGMKKYFVGVNAHGHVAISAKKIEGENIGAQVLGLFTLSTGQDSWQKLSGGGHHHHHH

SEQ ID NO: 29 - protein, 11 aa, Streptococcus pyogenes
PLTPEQFRYNN

SEQ ID NO: 30 - protein, 8 aa, Streptococcus pyogenes
PPANFTQG

SEQ ID NO: 31 - protein, 20 aa, Streptococcus pyogenes
DDYQRNATEAYAKEVPHQIT

SEQ ID NO: 32 - protein, 20 aa, Streptococcus pyogenes
DSFSANQEIRYSEVTPYHVT

SEQ ID NO: 33 - DNA, 963 bp, Streptococcus pyogenes
atggatagtttttctgctaatcaagagattagatattcggaagtaacaccttatcacgttacttccgtttggaccaaaggagttactcctccagcaaacttcactcaaggtgaagatgtttttcacgctccttatgttgctaaccaaggatggtatgatattaccaaaacattcaatggaaaagacgatcttctttgcggggctgccacagcagggaatatgcttcactggtggttcgatcaaaacaaagaccaaattaaacgttatttggaagagcatccagaaaagcaaaaaataaacttcaatggcgaacagatgtttgacgtaaaagaagctatcgacactaaaaaccaccagctagatagtaaattatttgaatattttaaagaaaaagctttcccttatctatctactaaacacctaggagttttccctgatcatgtaattgatatgttcattaacggctaccgccttagtctaactaaccacggtccaacgccagtaaaagaaggtagtaaagatccccgaggtggtatttttgacgccgtatttacaagaggtgatcaaagtaagctattgacaagtcgtcatgattttaaagaaaaaaatctcaaagaaatcagtgatctcattaagaaagagttaaccgaaggcaaggctctaggcctatcacacacctacgctaacgtacgcatcaaccatgttataaacctgtggggagctgactttgattctaacgggaaccttaaagctatttatgtaacagactctgatagtaatgcatctattggtatgaagaaatactttgttggtgttaattccgctggaaaagtagctatttctgctaaagaaataaaagaagataatataggtgctcaagtactagggttatttacactttcaacagggcaagatagttggaatcagaccaatggcggtggccatcatcaccatcaccactaa

SEQ ID NO: 34 - DNA, 978 bp, Streptococcus pyogenes
atggacgattaccaaaggaatgctacggaagcttatgccaaagaagtaccacatcagatcacttctgtatggaccaaaggtgttacaccactaacacccgagcagtttcgatataataacgaagatgtgatccatgcgccatatcttgctcatcaaggctggtacgatatcaccaaggccttcgatgggaaggataatctcttgtgtggcgcagcaacggcaggtaatatgctgcattggtggtttgatcaaaataaaacagagattgaagcctatttaagtaaacaccctgaaaagcaaaaaatcatttttaacaaccaagagctatttgatttgaaagctgctatcgataccaaggacagtcaaaccaatagtcagctttttaattattttagagataaagcctttccaaatctatcagcacgtcaactcggggttatgcctgatcttgttctagatatgtttatcaatggttactacttaaatgtgtttaaaacacagtctactgatgtcaatcgaccttatcaggacaaggacaaacgaggtggtattttcgatgctgttttcaccagaggagatcagacaacgctcttgacagctcgtcatgatttaaaaaataaaggactaaatgacatcagcaccattatcaagcaagaactgactgaaggaagagcccttgctttatcacatacctacgccaatgttagcattagccatgtgattaacttgtggggagctgattttaatgctgaaggaaaccttgaggccatctatgtcacagactcagatgctaatgcgtctattggtatgaaaaaatattttgtcggcattaatgctcatggacatgtcgccatttctgccaagaaaatagaaggagaaaacattggcgctcaagtattaggcttatttacgctttccagtggcaaggacatttggcagaaactgagcggcggtggccatcatcaccatcaccactaa

SEQ ID NO: 35 - DNA, 972 bp, Streptococcus pyogenes
atggatgattatcagcgcaacgcgaccgaagcgtatgcgaaagaagtgccgcatcagattaccagcgtgtggaccaaaggcgtgaccccgctgaccccggaacagtttcgctataacaacgaagatgtgtttcatgcgccgtatgtggcgaaccagggctggtatgatattaccaaagcgtttgatggcaaagataacctgctgtgcggcgcggcgaccgcgggcaacatgctgcattggtggtttgatcagaacaaagatcagattaaacgctatctggaagaacatccggaaaaacagaaaattaactttaacggcgataacatgtttgatgtgaaaaaagcgattgataccaaaaaccatcagctggatagcaaactgtttaactattttaaagaaaaagcgtttccgggcctgagcgcgcgccgcattggcgtgtttccggatcatgtgattgatatgtttattaacggctatcgcctgagcctgaccaaccatggcccgaccccggtgaaagaaggcagcaaagatccgcgcggcggcatttttgatgcggtgtttacccgcggcaaccagagcaaactgctgaccagccgccatgattttaaaaacaaaaacctgaacgatattagcaccattattaaacaggaactgaccaaaggcaaagcgctgggcctgagccatacctatgcgaacgtgagcattaaccatgtgattaacctgtggggcgcggattttaacgcggaaggcaacctggaagcgatttatgtgaccgatagcgatagcaacgcgagcattggcatgaaaaaatattttgtgggcgtgaacgcgcatggccatgtggcgattagcgcgaaaaaaattgaaggcgaaaacattggcgcgcaggtgctgggcctgtttaccctgagcaccggccaggatagctggcagaaactgagcggcggtggccatcatcaccatcaccactaa

SEQ ID NO: 36 - DNA, 978 bp, Streptococcus pyogenes
atggatgattatcagcgcaacgcgaccgaagcgtatgcgaaagaagtgccgcatcagattaccagcgtgtggaccaaaggcgtgaccccgctgaccccggaacagtttcgctataacaacgaagatgtgattcatgcgccgtatctggcgaaccagggctggtatgatattaccaaagcgtttgatggcaaagataacctgctgtgcggcgcggcgaccgcgggcaacatgctgcattggtggtttgatcagaacaaaaccgaaattgaagcgtatctgagcaaacatccggaaaaacagaaaattatttttcgcaaccaggaactgtttgatctgaaagaagcgattcgcaccaaagatagccagaccaacagccagctgtttgaatattttcgcgataaagcgtttccgtatctgagcgcgcgccagctgggcgtgatgccggatctggtgctggatatgtttattaacggctattatctgaacgtgtttaaaacccagagcaccgatgtgaaacgcccgtatcaggataaagataaacgcggcggcatttttgatgcggtgtttacccgcggcaaccagaccaccctgctgaccgcgcgccatgatctgaaaaacaaaggcctgaacgatattagcaccattattaaagaagaactgaccaaaggccgcgcgctggcgctgagccatacctatgcgaacgtgagcattagccatgtgattaacctgtggggcgcggattttaacgcggaaggcaacctggaagcgatttatgtgaccgatagcgatgcgaacgcgagcattggcatgaaaaaatattttgtgggcattaacaaacatggccatgtggcgattagcgcgaaaaaaattgaaggcgaaaacattggcgcgcaggtgctgggcctgtttaccctgagcagcggcaaagatatttggcagaaactgaacggcggtggccatcatcaccatcaccactaa

SEQ ID NO: 37 - DNA, 978 bp, Streptococcus pyogenes
atggatgattatcagcgcaacgcgaccgaagcgtatgcgaaagaagtgccgcatcagattaccagcgtgtggaccaaaggcgtgaccccgctgaccccggaacagtttcgctataacaacgaagatgtgattcatgcgccgtatctggcgcatcagggctggtatgatattaccaaaacctttaacggcaaagataacctgctgtgcggcgcggcgaccgcgggcaacatgctgcattggtggtttgatcagaacaaaaccgaaattgaagcgtatctgagcaaacatccggaaaaacagaaaattatttttaacaacgaagaactgtttgatctgaaagcggcgattgataccaaagatagccagaccaacagccagctgtttaactattttaaagaaaaagcgtttccgaacctgagcacccgccagctgggcgtgatgccggatctggtgctggatatgtttattaacggctattatctgaacgtgtttaaaacccagagcaccgatgtgaaccgcccgtatcaggataaagataaacgcggcggcatttttgatgcggtgtttacccgcggcaaccagaccaccctgctgaccgcgcgccatgattttaaagaaaaaggcctgaaagatattagcaccattattaaacaggaactgaccgaaggccgcgcgctggcgctgagccatacctatgcgaacgtgagcattagccatgtgattaacctgtggggcgcggattttgatgcggaaggcaacctgaaagcgatttatgtgaccgatagcgatgcgaacgcgagcattggcatgaaaaaatattttgtgggcattaacgcgcatggcaaagtggcgattagcgcgaaaaaaattgaaggcgaaaacattggcgcgcaggtgctgggcctgtttaccctgagcagcggcaaagatatttggcagcagctgagcggcggtggccatcatcaccatcaccactaa

SEQ ID NO: 38 - DNA, 978 bp, Streptococcus pyogenes
atggatagctttagcgcgaaccaggaaattcgctatagcgaagtgaccccgtatcatgtgaccagcgtgtggaccaaaggcgtgaccccgctgaccccggaacagtttcgctataacaacgaagatgtgattcatgcgccgtatctggcgcatcagggctggtatgatattaccaaagcgtttgatggcaaagataacctgctgtgcggcgcggcgaccgcgggcaacatgctgcattggtggtttgatcagaacaaaaccgaaattgaagcgtatctgagcaaacatccggaaaaacagaaaattatttttaacaaccaggaactgtttgatctgaaagcggcgattgataccaaagatagccagaccaacagccagctgtttaactattttcgcgataaagcgtttccgaacctgagcgcgcgccagctgggcgtgatgccggatctggtgctggatatgtttattaacggctattatctgaacgtgtttaaaacccagagcaccgatgtgaaccgcccgtatcaggataaagataaacgcggcggcatttttgatgcggtgtttacccgcggcgatcagaccaccctgctgaccgcgcgccatgatctgaaaaacaaaggcctgaacgatattagcaccattattaaacaggaactgaccgaaggccgcgcgctggcgctgagccatacctatgcgaacgtgagcattagccatgtgattaacctgtggggcgcggattttaacgcggaaggcaacctggaagcgatttatgtgaccgatagcgatgcgaacgcgagcattggcatgaaaaaatattttgtgggcattaacgcgcatggccatgtggcgattagcgcgaaaaaaattgaaggcgaaaacattggcgcgcaggtgctgggcctgtttaccctgagcagcggcaaagatatttggcagaaactgagcggcggtggccatcatcaccatcaccactaa

SEQ ID NO: 39 - DNA, 918 bp, Streptococcus pyogenes
atgagcgtgtggaccaaaggcgtgaccccgctgaccccggaacagtttcgctataacaacgaagatgtgattcatgcgccgtatctggcgcatcagggctggtatgatattaccaaagcgtttgatggcaaagataacctgctgtgcggcgcggcgaccgcgggcaacatgctgcattggtggtttgatcagaacaaaaccgaaattgaagcgtatctgagcaaacatccggaaaaacagaaaattatttttaacaaccaggaactgtttgatctgaaagcggcgattgataccaaagatagccagaccaacagccagctgtttaactattttcgcgataaagcgtttccgaacctgagcgcgcgccagctgggcgtgatgccggatctggtgctggatatgtttattaacggctattatctgaacgtgtttaaaacccagagcaccgatgtgaaccgcccgtatcaggataaagataaacgcggcggcatttttgatgcggtgtttacccgcggcgatcagaccaccctgctgaccgcgcgccatgatctgaaaaacaaaggcctgaacgatattagcaccattattaaacaggaactgaccgaaggccgcgcgctggcgctgagccatacctatgcgaacgtgagcattagccatgtgattaacctgtggggcgcggattttaacgcggaaggcaacctggaagcgatttatgtgaccgatagcgatgcgaacgcgagcattggcatgaaaaaatattttgtgggcattaacgcgcatggccatgtggcgattagcgcgaaaaaaattgaaggcgaaaacattggcgcgcaggtgctgggcctgtttaccctgagcagcggcaaagatatttggcagaaactgagcggcggtggccatcatcaccatcaccactaa

SEQ ID NO: 40 - DNA, 975 bp, Streptococcus pyogenes
atggacgattaccaaaggaatgctacggaagcttatgccaaagaagtaccacatcagatcacttctgtatggaccaaaggtgttacaccactaacacccgagcagtttactcaaggtgaagatgtgatccatgcgccatatcttgctcatcaaggctggtacgatatcaccaaggccttcgatgggaaggataatctcttgtgtggcgcagcaacggcaggtaatatgctgcattggtggtttgatcaaaataaaacagagattgaagcctatttaagtaaacaccctgaaaagcaaaaaatcatttttaacaaccaagagctatttgatttgaaagctgctatcgataccaaggacagtcaaaccaatagtcagctttttaattattttagagataaagcctttccaaatctatcagcacgtcaactcggggttatgcctgatcttgttctagatatgtttatcaatggttactacttaaatgtgtttaaaacacagtctactgatgtcaatcgaccttatcaggacaaggacaaacgaggtggtattttcgatgctgttttcaccagaggagatcagacaacgctcttgacagctcgtcatgatttaaaaaataaaggactaaatgacatcagcaccattatcaagcaagaactgactgaaggaagagcccttgctttatcacatacctacgccaatgttagcattagccatgtgattaacttgtggggagctgattttaatgctgaaggaaaccttgaggccatctatgtcacagactcagatgctaatgcgtctattggtatgaaaaaatattttgtcggcattaatgctcatggacatgtcgccatttctgccaagaaaatagaaggagaaaacattggcgctcaagtattaggcttatttacgctttccagtggcaaggacatttggcagaaactgagcggcggtggccatcatcaccatcaccactaa

SEQ ID NO: 41 - DNA, 969 bp, Streptococcus pyogenes
atggacgattaccaaaggaatgctacggaagcttatgccaaagaagtaccacatcagatcacttctgtatggaccaaaggtgttacaccacccgagcagtttactcaaggtgaagatgtgatccatgcgccatatcttgctcatcaaggctggtacgatatcaccaaggccttcgatgggaaggataatctcttgtgtggcgcagcaacggcaggtaatatgctgcattggtggtttgatcaaaataaaacagagattgaagcctatttaagtaaacaccctgaaaagcaaaaaatcatttttaacaaccaagagctatttgatttgaaagctgctatcgataccaaggacagtcaaaccaatagtcagctttttaattattttagagataaagcctttccaaatctatcagcacgtcaactcggggttatgcctgatcttgttctagatatgtttatcaatggttactacttaaatgtgtttaaaacacagtctactgatgtcaatcgaccttatcaggacaaggacaaacgaggtggtattttcgatgctgttttcaccagaggagatcagacaacgctcttgacagctcgtcatgatttaaaaaataaaggactaaatgacatcagcaccattatcaagcaagaactgactgaaggaagagcccttgctttatcacatacctacgccaatgttagcattagccatgtgattaacttgtggggagctgattttaatgctgaaggaaaccttgaggccatctatgtcacagactcagatgctaatgcgtctattggtatgaaaaaatattttgtcggcattaatgctcatggacatgtcgccatttctgccaagaaaatagaaggagaaaacattggcgctcaagtattaggcttatttacgctttccagtggcaaggacatttggcagaaactgagcggcggtggccatcatcaccatcaccactaa

SEQ ID NO: 42 - DNA, 972 bp, Streptococcus pyogenes
atggacgattaccaaaggaatgctacggaagcttatgccaaagaagtaccacatcagatcacttctgtatggaccaaaggtgttacaccacccgagcagtttcgatataataacgaagatgtgatccatgcgccatatcttgctcatcaaggctggtacgatatcaccaaggccttcgatgggaaggataatctcttgtgtggcgcagcaacggcaggtaatatgctgcattggtggtttgatcaaaataaaacagagattgaagcctatttaagtaaacaccctgaaaagcaaaaaatcatttttaacaaccaagagctatttgatttgaaagctgctatcgataccaaggacagtcaaaccaatagtcagctttttaattattttagagataaagcctttccaaatctatcagcacgtcaactcggggttatgcctgatcttgttctagatatgtttatcaatggttactacttaaatgtgtttaaaacacagtctactgatgtcaatcgaccttatcaggacaaggacaaacgaggtggtattttcgatgctgttttcaccagaggagatcagacaacgctcttgacagctcgtcatgatttaaaaaataaaggactaaatgacatcagcaccattatcaagcaagaactgactgaaggaagagcccttgctttatcacatacctacgccaatgttagcattagccatgtgattaacttgtggggagctgattttaatgctgaaggaaaccttgaggccatctatgtcacagactcagatgctaatgcgtctattggtatgaaaaaatattttgtcggcattaatgctcatggacatgtcgccatttctgccaagaaaatagaaggagaaaacattggcgctcaagtattaggcttatttacgctttccagtggcaaggacatttggcagaaactgagcggcggtggccatcatcaccatcaccactaa

SEQ ID NO: 43 - DNA, 969 bp, Streptococcus pyogenes
atggacgattaccaaaggaatgctacggaagcttatgccaaagaagtaccacatcagatcacttctgtatggaccaaaggtgttacaccacccgagcagtttactcaaggtgaagatgtgatccatgcgccatatcttgctcatcaaggctggtacgatatcaccaaggccttcgatgggaaggataatctcttgtgtggcgcagcaacggcaggtaatatgctgcattggtggtttgatcaaaataaaacagagattgaagcctatttaagtaaacaccctgaaaagcaaaaaatcattattaacaaccaagagctatttgatttgaaagctgctatcgataccaaggacagtcaaaccaatagtcagctttttaattattttagagataaagcctttccaaatctatcagcacgtcaactcggggttatgcctgatcttgttctagatatgtttatcaatggttactacttaaatgtgtttaaaacacagtctactgatgtcaatcgaccttatcaggacaaggacaaacgaggtggtattttcgatgctgttttcaccagaggagatcagacaacgctcttgacagctcgtcatgatttaaaaaataaaggactaaatgacatcagcaccattatcaagcaagaactgactgaaggaagagcccttgctttatcacatacctacgccaatgttagcattagccatgtgattaacttgtggggagctgattttaatgctgaaggaaaccttgaggccatctatgtcacagactcagatgctaatgcgtctattggtatgaaaaaatattttgtcggcattaatgctcatggacatgtcgccatttctgccaagaaaatagaaggagaaaacattggcgctcaagtattaggcttatttacgctttccagtggcaaggacatttggcagaaactgagcggcggtggccatcatcaccatcaccactaa

SEQ ID NO: 44 - DNA, 969 bp, Streptococcus pyogenes
atggacgattaccaaaggaatgctacggaagcttatgccaaagaagtaccacatcagatcacttctgtatggaccaaaggtgttacaccacccgagcagtttactcaaggtgaagatgtgatccatgcgccatatcttgctcatcaaggctggtacgatatcaccaaggccttcgatgggaaggataatctcttgtgtggcgcagcaacggcaggtaatatgctgcattggtggtttgatcaaaataaaacagagattgaagcctatttaagtaaacaccctgaaaagcaaaaaatcatttttcgtaaccaagagctatttgatttgaaagctgctatcgataccaaggacagtcaaaccaatagtcagctttttaattattttagagataaagcctttccaaatctatcagcacgtcaactcggggttatgcctgatcttgttctagatatgtttatcaatggttactacttaaatgtgtttaaaacacagtctactgatgtcaatcgaccttatcaggacaaggacaaacgaggtggtattttcgatgctgttttcaccagaggagatcagacaacgctcttgacagctcgtcatgatttaaaaaataaaggactaaatgacatcagcaccattatcaagcaagaactgactgaaggaagagcccttgctttatcacatacctacgccaatgttagcattagccatgtgattaacttgtggggagctgattttaatgctgaaggaaaccttgaggccatctatgtcacagactcagatgctaatgcgtctattggtatgaaaaaatattttgtcggcattaatgctcatggacatgtcgccatttctgccaagaaaatagaaggagaaaacattggcgctcaagtattaggcttatttacgctttccagtggcaaggacatttggcagaaactgagcggcggtggccatcatcaccatcaccactaa

SEQ ID NO: 45 - DNA, 969 bp, Streptococcus pyogenes
atggacgattaccaaaggaatgctacggaagcttatgccaaagaagtaccacatcagatcacttctgtatggaccaaaggtgttacaccacccgagcagtttactcaaggtgaagatgtgatccatgcgccatatcttgctcatcaaggctggtacgatatcaccaaggccttcgatgggaaggataatctcttgtgtggcgcagcaacggcaggtaatatgctgcattggtggtttgatcaaaataaaacagagattgaagcctatttaagtaaacaccctgaaaagcaaaaaatcattattcgtaaccaagagctatttgatttgaaagctgctatcgataccaaggacagtcaaaccaatagtcagctttttaattattttagagataaagcctttccaaatctatcagcacgtcaactcggggttatgcctgatcttgttctagatatgtttatcaatggttactacttaaatgtgtttaaaacacagtctactgatgtcaatcgaccttatcaggacaaggacaaacgaggtggtattttcgatgctgttttcaccagaggagatcagacaacgctcttgacagctcgtcatgatttaaaaaataaaggactaaatgacatcagcaccattatcaagcaagaactgactgaaggaagagcccttgctttatcacatacctacgccaatgttagcattagccatgtgattaacttgtggggagctgattttaatgctgaaggaaaccttgaggccatctatgtcacagactcagatgctaatgcgtctattggtatgaaaaaatattttgtcggcattaatgctcatggacatgtcgccatttctgccaagaaaatagaaggagaaaacattggcgctcaagtattaggcttatttacgctttccagtggcaaggacatttggcagaaactgagcggcggtggccatcatcaccatcaccactaa

SEQ ID NO: 46 - DNA, 969 bp, Streptococcus pyogenes
atggatgattatcagcgcaacgcgaccgaagcgtatgcgaaagaagtgccgcatcagattaccagcgtgtggaccaaaggcgtgaccccgccggaacagtttactcaaggtgaagatgtgattcatgcgccgtatctggcgaaccagggctggtatgatattaccaaagcgtttgatggcaaagataacctgctgtgcggcgcggcgaccgcgggcaacatgctgcattggtggtttgatcagaacaaaaccgaaattgaagcgtatctgagcaaacatccggaaaaacagaaaattatttttcgcaaccaggaactgtttgatctgaaagaagcgattcgcaccaaagatagccagaccaacagccagctgtttgaatattttcgcgataaagcgtttccgtatctgagcgcgcgccagctgggcgtgatgccggatctggtgctggatatgtttattaacggctattatctgaacgtgtttaaaacccagagcaccgatgtgaaacgcccgtatcaggataaagataaacgcggcggcatttttgatgcggtgtttacccgcggcaaccagaccaccctgctgaccgcgcgccatgatctgaaaaacaaaggcctgaacgatattagcaccattattaaagaagaactgaccaaaggccgcgcgctggcgctgagccatacctatgcgaacgtgagcattagccatgtgattaacctgtggggcgcggattttaacgcggaaggcaacctggaagcgatttatgtgaccgatagcgatgcgaacgcgagcattggcatgaaaaaatattttgtgggcattaacaaacatggccatgtggcgattagcgcgaaaaaaattgaaggcgaaaacattggcgcgcaggtgctgggcctgtttaccctgagcagcggcaaagatatttggcagaaactgaacggcggtggccatcatcaccatcaccactaa

SEQ ID NO: 47 - DNA, 909 bp, Streptococcus pyogenes
atgtctgtatggaccaaaggtgttacaccacccgagcagtttactcaaggtgaagatgtgatccatgcgccatatcttgctcatcaaggctggtacgatatcaccaaggccttcgatgggaaggataatctcttgtgtggcgcagcaacggcaggtaatatgctgcattggtggtttgatcaaaataaaacagagattgaagcctatttaagtaaacaccctgaaaagcaaaaaatcatttttcgtaaccaagagctatttgatttgaaagctgctatcgataccaaggacagtcaaaccaatagtcagctttttaattattttagagataaagcctttccaaatctatcagcacgtcaactcggggttatgcctgatcttgttctagatatgtttatcaatggttactacttaaatgtgtttaaaacacagtctactgatgtcaatcgaccttatcaggacaaggacaaacgaggtggtattttcgatgctgttttcaccagaggaaaccagacaacgctcttgacagctcgtcatgatttaaaaaataaaggactaaatgacatcagcaccattatcaagcaagaactgactgaaggaagagcccttgctttatcacatacctacgccaatgttagcattagccatgtgattaacttgtggggagctgattttaatgctgaaggaaaccttgaggccatctatgtcacagactcagatgctaatgcgtctattggtatgaaaaaatattttgtcggcattaatgctcatggacatgtcgccatttctgccaagaaaatagaaggagaaaacattggcgctcaagtattaggcttatttacgctttccagtggcaaggacatttggcagaaactgagcggcggtggccatcatcaccatcaccactaa

SEQ ID NO: 48 - DNA, 969 bp, Streptococcus pyogenes
atggacgattaccaaaggaatgctacggaagcttatgccaaagaagtaccacatcagatcacttctgtatggaccaaaggtgttacaccacccgagcagtttactcaaggtgaagatgtgatccatgcgccatatcttgctcatcaaggctggtacgatatcaccaaggccttcgatggggcggataatctcttgtgtggcgcagcaacggcaggtaatatgctgcattggtggtttgatcaaaataaaacagagattgaagcctatttaagtaaacaccctgaaaagcaaaaaatcatttttcgtaaccaagagctatttgatttgaaagctgctatcgataccaaggacagtcaaaccaatagtcagctttttaattattttagagataaagcctttccaaatctatcagcacgtcaactcggggttatgcctgatcttgttctagatatgtttatcaatggttactacttaaatgtgtttaaaacacagtctactgatgtcaatcgaccttatcaggacaaggacaaacgaggtggtattttcgatgctgttttcaccagaggaaatcagacaacgctcttgacagctcgtcatgatttaaaaaataaaggactaaatgacatcagcaccattatcaagcaagaactgactgaaggaagagcccttgctttatcacatacctacgccaatgttagcattagccatgtgattaacttgtggggagctgattttaatgctgaaggaaaccttgaggccatctatgtcacagactcagatgctaatgcgtctattggtatgaaaaaatattttgtcggcattaatgctcatggacatgtcgccatttctgccaagaaaatagaaggagaaaacattggcgctcaagtattaggcttatttacgctttccagtggcaaggacatttggcagaaactgagcggcggtggccatcatcaccatcaccactaa

SEQ ID NO: 49 - DNA, 909 bp, Streptococcus pyogenes
atgtctgtatggaccaaaggtgttacaccacccgagcagtttactcaaggtgaagatgtgatccatgcgccatatcttgctcatcaaggctggtacgatatcaccaaggccttcgatggggcggataatctcttgtgtggcgcagcaacggcaggtaatatgctgcattggtggtttgatcaaaataaaacagagattgaagcctatttaagtaaacaccctgaaaagcaaaaaatcatttttcgtaaccaagagctatttgatttgaaagctgctatcgataccaaggacagtcaaaccaatagtcagctttttaattattttagagataaagcctttccaaatctatcagcacgtcaactcggggttatgcctgatcttgttctagatatgtttatcaatggttactacttaaatgtgtttaaaacacagtctactgatgtcaatcgaccttatcaggacaaggacaaacgaggtggtattttcgatgctgttttcaccagaggaaatcagacaacgctcttgacagctcgtcatgatttaaaaaataaaggactaaatgacatcagcaccattatcaagcaagaactgactgaaggaagagcccttgctttatcacatacctacgccaatgttagcattagccatgtgattaacttgtggggagctgattttaatgctgaaggaaaccttgaggccatctatgtcacagactcagatgctaatgcgtctattggtatgaaaaaatattttgtcggcattaatgctcatggacatgtcgccatttctgccaagaaaatagaaggagaaaacattggcgctcaagtattaggcttatttacgctttccagtggcaaggacatttggcagaaactgagcggcggtggccatcatcaccatcaccactaa

SEQ ID NO: 50 - DNA, 969 bp, Streptococcus pyogenes
atggacgattaccaaaggaatgctacggaagcttatgccaaagaagtaccacatcagatcacttctgtatggaccaaaggtgttacaccacccgagcagtttactcaaggtgaagatgtgatccatgcgccatatcttgctcatcaaggctggtacgatatcaccaaggccttcgatgggaaggataatctcttgtgtggcgcagcaacggcaggtaatatgctgcattggtggtttgatcaaaataaaacagagattgaagcctatttaagtaaacaccctgaaaagcaaaaaatcatttttcgtaaccaagagctatttgatttgaaagctgctatcgataccaaggacagtcaaaccaatagtcagctttttaattattttagagataaagcctttccaaatctatcagcacgtcaactcggggttatgcctgatcttgttctagatatgtttatcaatggttactacttaaatgtgtttaaaacacagtctactgatgtcaatcgaccttatcaggacaaggacaaacgaggtggtattttcgatgctgttttcaccagaggaaaccagacaacgctcttgacagctcgtcatgatttaaaaaataaaggactaaatgacatcagcaccattatcaagcaagaactgactgaaggaagagcccttgctttatcacatacctacgccaatgttagcattagccatgtgattaacttgtggggagctgattttaatgctgaaggaaaccttgaggccatctatgtcacagactcagatgctaatgcgtctattggtatgaaaaaatattttgtcggcattaatgctcatggacatgtcgccatttctgccaagaaaatagaaggagaaaacattggcgctcaagtattaggcttatttacgctttccagtggcaaggacatttggcagaaactgagcggcggtggccatcatcaccatcaccactaa

SEQ ID NO: 51 - DNA, 969 bp, Streptococcus pyogenes
atggatgattatcagcgcaacgcgaccgaagcgtatgcgaaagaagtgccgcatcagattaccagcgtgtggaccaaaggcgtgaccccgctgaccccggaacagtttacccagggcgaagatgtgtttcatgcgccgtatgtggcgaaccagggctggtatgatattaccaaagcgtttgatggcaaagataacctgctgtgcggcgcggcgaccgcgggcaacatgctgcattggtggtttgatcagaacaaagatcagattaaacgctatctggaagaacatccggaaaaacagaaaattaactttaacggcgaaaacatgtttgatgtgaaaaaagcgattgataccaaaaaccatcagctggatagcaaactgtttaactattttaaagaaaaagcgtttccgtatctgagcgcgaaacatctgggcgtgtttccggatcatgtgattgatatgtttattaacggctatcgcctgagcctgaccaaccatggcccgaccccggtgaaagaaggcagcaaagatccgcgcggcggcatttttgatgcggtgtttacccgcggcaaccagagcaaactgctgaccagccgccatgattttaaaaacaaaaacctgaacgatattagcaccattattaaacaggaactgaccaaaggcaaagcgctgggcctgagccatacctatgcgaacgtgcgcattaaccatgtgattaacctgtggggcgcggattttaacgcggaaggcaacctggaagcgatttatgtgaccgatagcgatagcaacgcgagcattggcatgaaaaaatattttgtgggcgtgaacgcgcatggccatgtggcgattagcgcgaaaaaaattgaaggcgaaaacattggcgcgcaggtgctgggcctgtttaccctgagcaccggccaggatagctggcagaaactgagcggcggtggccatcatcaccatcaccactaa

SEQ ID NO: 52 - DNA, 969 bp, Streptococcus pyogenes
atggatgattatcagcgcaacgcgaccgaagcgtatgcgaaagaagtgccgcatcagattaccagcgtgtggaccaaaggcgtgaccccgctgaccccggaacagtttacccagggcgaagatgtgtttcatgcgccgtatgtggcgaaccagggctggtatgatattaccaaagcgtttgatggcaaagataacctgctgtgcggcgcggcgaccgcgggcaacatgctgcattggtggtttgatcagaacaaagatcagattaaacgctatctggaagaacatccggaaaaacagaaaattaactttcgcggcgaaaacatgtttgatgtgaaagaagcgattcgcaccaaaaaccatcagctggatagcaaactgtttgaatattttaaagaaaaagcgtttccgtatctgagcgcgaaacatctgggcgtgtttccggatcatgtgattgatatgtttattaacggctatcgcctgagcctgaccaaccatggcccgaccccggtgaaaaaaggcagcaaagatccgcgcggcggcatttttgatgcggtgtttacccgcggcaaccagagcaaactgctgaccagccgccatgattttaaaaacaaaaacctgaacgatattagcaccattattaaaagcgaactgaccaacggcaaagcgctgggcctgagccatacctatgcgaacgtgcgcattaaccatgtgattaacctgtggggcgcggattttaacgcggaaggcaacctggaagcgatttatgtgaccgatagcgatagcaacgcgagcattggcatgaaaaaatattttgtgggcgtgaacaaacatggccatgtggcgattagcgcgaaaaaaattgaaggcgaaaacattggcgcgcaggtgctgggcctgtttaccctgagcaccggccaggatagctggcagaaactgaacggcggtggccatcatcaccatcaccactaa

SEQ ID NO: 53 - DNA, 969 bp, Streptococcus pyogenes
atggatgattatcagcgcaacgcgaccgaagcgtatgcgaaagaagtgccgcatcagattaccagcgtgtggaccaaaggcgtgaccccgctgaccccggaacagtttacccagggcgaagatgtgtttcatgcgccgtatgtggcgaaccagggctggtatgatattaccaaaacctttaacggcaaagatgatctgctgtgcggcgcggcgaccgcgggcaacatgctgcattggtggtttgatcagaacaaagatcagattaaacgctatctggaagaacatccggaaaaacagaaaattaactttaacggcgaacagatgtttgatgtgaaagaagcgattgataccaaaaaccatcagctggatagcaaactgtttgaatattttaaagaaaaagcgtttccgtatctgagcaccaaacatctgggcgtgtttccggatcatgtgattgatatgtttattaacggctatcgcctgagcctgaccaaccatggcccgaccccggtgaaagaaggcagcaaagatccgcgcggcggcatttttgatgcggtgtttacccgcggcaaccagagcaaactgctgaccagccgccatgattttaaagaaaaaaacctgaaagaaattagcgatctgattaaacaggaactgaccgaaggcaaagcgctgggcctgagccatacctatgcgaacgtgcgcattaaccatgtgattaacctgtggggcgcggattttgatgcggaaggcaacctgaaagcgatttatgtgaccgatagcgatagcaacgcgagcattggcatgaaaaaatattttgtgggcgtgaacgcggcgggcaaagtggcgattagcgcgaaaaaaattgaaggcgaaaacattggcgcgcaggtgctgggcctgtttaccctgagcaccggccaggatagctggaaccagaccagcggcggtggccatcatcaccatcaccactaa

SEQ ID NO: 54 - DNA, 969 bp, Streptococcus pyogenes
atggatgattatcagcgcaacgcgaccgaagcgtatgcgaaagaagtgccgcatcagattaccagcgtgtggaccaaaggcgtgaccccgctgaccccggaacagtttacccagggcgaagatgtgtttcatgcgccgtatgtggcgaaccagggctggtatgatattaccaaaacctttaacggcaaagatgatctgctgtgcggcgcggcgaccgcgggcaacatgctgcattggtggtttgatcagaacaaagatcagattaaacgctatctggaagaacatccggaaaaacagaaaattaactttcgcggcgaacagatgtttgatgtgaaagaagcgattcgcaccaaaaaccatcagctggatagcaaactgtttgaatattttaaagaaaaagcgtttccgtatctgagcaccaaacatctgggcgtgtttccggatcatgtgattgatatgtttattaacggctatcgcctgagcctgaccaaccatggcccgaccccggtgaaaaaaggcagcaaagatccgcgcggcggcatttttgatgcggtgtttacccgcggcaaccagagcaaactgctgaccagccgccatgattttaaagaaaaaaacctgaaagaaattagcgatctgattaaagaagaactgaccaaaggcaaagcgctgggcctgagccatacctatgcgaacgtgcgcattaaccatgtgattaacctgtggggcgcggattttgatgcggaaggcaacctgaaagcgatttatgtgaccgatagcgatagcaacgcgagcattggcatgaaaaaatattttgtgggcgtgaacaaagcgggcaaagtggcgattagcgcgaaaaaaattgaaggcgaaaacattggcgcgcaggtgctgggcctgtttaccctgagcaccggccaggatagctggaaccagaccaacggcggtggccatcatcaccatcaccactaa

SEQ ID NO: 55 - DNA, 963 bp, Streptococcus pyogenes
atggatgattatcagcgcaacgcgaccgaagcgtatgcgaaagaagtgccgcatcagattaccagcgtgtggaccaaaggcgtgaccccgccggaacagtttactcaaggtgaagatgtgattcatgcgccgtatgtggcgaaccagggctggtatgatattaccaaagcgtttgatggcaaagataacctgctgtgcggcgcggcgaccgcgggcaacatgctgcattggtggtttgatcagaacaaagatcagattaaacgctatctggaagaacatccggaaaaacagaaaattaactttcgcggcgaacagatgtttgatgtgaaaaaagcgattgataccaaaaaccatcagctggatagcaaactgtttaactattttaaagaaaaagcgtttccgggcctgagcgcgcgccgcattggcgtgtttccggatcatgtgattgatatgtttattaacggctatcgcctgagcctgaccaaccatggcccgaccccggtgaaagaaggcagcaaagatccgcgcggcggcatttttgatgcggtgtttacccgcggcaaccagagcaaactgctgaccagccgccatgattttaaaaacaaaaacctgaacgatattagcaccattattaaacaggaactgaccaaaggcaaagcgctgggcctgagccatacctatgcgaacgtgagcattaaccatgtgattaacctgtggggcgcggattttaacgcggaaggcaacctggaagcgatttatgtgaccgatagcgatagcaacgcgagcattggcatgaaaaaatattttgtgggcgtgaacgcgcatggccatgtggcgattagcgcgaaaaaaattgaaggcgaaaacattggcgcgcaggtgctgggcctgtttaccctgagcaccggccaggatagctggcagaaactgagcggcggtggccatcatcaccatcaccactaa